European Patent Application EP 4 772 529 A1, published July 8, 2026. Title: Peptide Having Activity of Skin Whitening and Uses Thereof. Applicant: CAREGEN CO., LTD. The sequence listing filed with the application follows.

SEQUENCE LISTING (7 sequences)

SEQ ID NO: 1 - protein, 10 aa, synthetic construct
KLKKDRMQRS

SEQ ID NO: 2 - DNA, 20 bp, synthetic construct
  source 1..20: mol_type = other DNA
gccgtctatttgccacacac

SEQ ID NO: 3 - DNA, 20 bp, synthetic construct
  source 1..20: mol_type = other DNA
gcagtcagcaacttcatggc

SEQ ID NO: 4 - DNA, 20 bp, synthetic construct
  source 1..20: mol_type = other DNA
tgaccaaacgtatccccctg

SEQ ID NO: 5 - DNA, 20 bp, synthetic construct
  source 1..20: mol_type = other DNA
ggtgtctgccgttgaagaga

SEQ ID NO: 6 - DNA, 20 bp, synthetic construct
  source 1..20: mol_type = other DNA
ggagccaaaagggtcatcat

SEQ ID NO: 7 - DNA, 20 bp, synthetic construct
  source 1..20: mol_type = other DNA
gtgatggcatggactgtggt